European Patent Application EP 4 155 315 A1, published March 29, 2023. Title: Matiple antigen peptide against corona virus and composition cmprising the same. Applicant: RIKEN Animal Allergy Clinical Laboratories. The sequence listing filed with the application follows.

SEQUENCE LISTING (8 sequences)

SEQ ID NO: 1 - protein, 11 aa, Artificial Sequence
  SARS-CoV-2 antigen peptide
SFIEDLLFNKV

SEQ ID NO: 2 - protein, 11 aa, Artificial Sequence
  FIPV antigen peptide
SAIEDLLFDKV

SEQ ID NO: 3 - protein, 31 aa, Artificial Sequence
  SARS-CoV-2 antigen peptide L
LPDPSKPSKRSFIEDLLFNKVTLADAGFIKQ

SEQ ID NO: 4 - protein, 25 aa, Artificial Sequence
  SARS-CoV-2 antigen peptide embeded in beta-sheet peptide
DRSFIEDLLFNKVGKGSIDTSAKFS

SEQ ID NO: 5 - protein, 25 aa, Artificial Sequence
  Influenza antigen peptide
DGWYGFRHQNSEGTGQAADLKSTQA

SEQ ID NO: 6 - protein, 11 aa, Artificial Sequence
  PEDV antigen peptide
SVIEDLLFNKV

SEQ ID NO: 7 - protein, 11 aa, Artificial Sequence
  Antigen peptide
  MISC_FEATURE (2)..(2): X = V, A, or F
  MISC_FEATURE (9)..(9): X = D or N
SXIEDLLFXKV

SEQ ID NO: 8 - protein, 11 aa, Artificial Sequence
  Peptide antigen
SAIEDLLFNKV